European Patent Specification EP 4 178 986 B1, published July 1, 2026. Title: Downregulation of Membrane-Bound Proteins by Receptor TAC Technology. Applicant: SHANDONG BOAN BIOTECHNOLOGY CO., LTD. Boan Boston LLC. The sequence listing filed with the application follows.

SEQUENCE LISTING (91 sequences)

SEQ ID NO: 1 - protein, 242 aa, Artificial Sequence
  CD19 CAR scFv
DIQMTQTTSSLSASLGDRVTISCRASQDISKYLNWYQQKPDGTVKLLIYHTSRLHSGVPSRFSGSGSGTDYSLTISNLEQEDIATYFCQQGNTLPYTFGGGTKLEITGGGGSGGGGSGGGGSEVKLQESGPGLVAPSQSLSVTCTVSGVSLPDYGVSWIRQPPRKGLEWLGVIWGSETTYYNSALKSRLTIIKDNSKSQVFLKMNSLQTDDTAIYYCAKHYYYGGSYAMDYWGQGTSVTVSS

SEQ ID NO: 2 - protein, 254 aa, Artificial Sequence
  SP34 scFv
EVQLVESGGGLVQPGGSLKLSCAASGFTFNKYAMNWVRQAPGKGLEWVARIRSKYNNYATYYADSVKDRFTISRDDSKNTAYLQMNNLKTEDTAVYYCVRHGNFGNSYISYWAYWGQGTLVTVSSGGGGSGGGGSGGGGSGGGGSQTVVTQEPSLTVSPGGTVTLTCGSSTGAVTSGYYPNWVQQKPGQAPRGLIGGTKFLAPGTPARFSGSLLGGKAALTLSGVQPEDEAEYYCALWYSNRWVFGGGTKLTVL

SEQ ID NO: 3 - protein, 241 aa, Artificial Sequence
  OKT3 scFv
QVQLVQSGGGVVQPGRSLRLSCKASGYTFTRYTMHWVRQAPGKGLEWIGYINPSRGYTNYNQKFKDRFTISRDNSKNTAFLQMDSLRPEDTGVYFCARYYDDHYSLDYWGQGTPVTVSSGGGGSGGGGSGGGGSDIQMTQSPSSLSASVGDRVTITCSASSSVSYMNWYQQTPGKAPKRWIYDTSKLASGVPSRFSGSGSGTDYTFTISSLQPEDIATYYCQQWSSNPFTFGQGTKLQITR

SEQ ID NO: 4 - protein, 250 aa, Artificial Sequence
  UCHT1 scFv
MDIQMTQTTSSLSASLGDRVTISCRASQDIRNYLNWYQQKPDGTVKLLIYYTSRLHSGVPSKFSGSGSGTDYSLTISNLEQEDIATYFCQQGNTLPWTFAGGTKLEIKGGGGSGGGGSGGGGSGGGGSEVQLQQSGPELVKPGASMKISCKASGYSFTGYTMNWVKQSHGKNLEWMGLINPYKGVSTYNQKFKDKATLTVDKSSSTAYMELLSLTSEDSAVYYCARSGYYGDSDWYFDVWGQGTTLTVFS

SEQ ID NO: 5 - protein, 245 aa, Artificial Sequence
  UCHT1.Y177T scFv
MDIQMTQSPSSLSASVGDRVTITCRASQDIRNYLNWYQQKPGKAPKLLIYYTSRLESGVPSRFSGSGSGTDYTLTISSLQPEDFATYYCQQGNTLPWTFGQGTKVEIKGGGGSGGGGSGGGGSEVQLVESGGGLVQPGGSLRLSCAASGYSFTGYTMNWVRQAPGKGLEWVALINPTKGVSTYNQKFKDRFTISVDKSKNTAYLQMNSLRAEDTAVYYCARSGYYGDSDWYFDVWGQGTLVTVSS

SEQ ID NO: 6 - protein, 240 aa, Artificial Sequence
  L2K scFv
DIQLTQSPAIMSASPGEKVTMTCRASSSVSYMNWYQQKSGTSPKRWIYDTSKVASGVPYRFSGSGSGTSYSLTISSMEAEDAATYYCQQWSSNPLTFGAGTKLELKGGGGSGGGGSGGGGSDIKLQQSGAELARPGASVKMSCKTSGYTFTRYTMHWVKQRPGQGLEWIGYINPSRGYTNYNQKFKDKATLTTDKSSSTAYMQLSSLTSEDSAVYYCARYYDDHYCLDYWGQGTTLTVSS

SEQ ID NO: 7 - protein, 249 aa, Artificial Sequence
  F6A scFv
QTVVTQEPSLTVSPGGTVTLTCGSSTGAVTSGYYPNWVQQKPGQAPRGLIGGTKFLAPGTPARFSGSLLGGKAALTLSGVQPEDEAEYYCALWYSNRWVFGGGTKLTVLGGGGSGGGGSGGGGSEVQLLESGGGLVQPGGSLKLSCAASGFTFNIYAMNWVRQAPGKGLEWVARIRSKYNNYATYYADSVKSRFTISRDDSKNTAYLQMNNLKTEDTAVYYCVRHGNFGNSYVSFFAYWGQGTLVTVSS

SEQ ID NO: 8 - protein, 241 aa, Artificial Sequence
  BMA031 scFv(i.e. BMA031.wt scFv)
EVQLQQSGPELVKPGASVKMSCKASGYKFTSYVMHWVKQKPGQGLEWIGYINPYNDVTKYNEKFKGKATLTSDKSSSTAYMELSSLTSEDSAVHYCARGSYYDYDGFVYWGQGTLVTVSAGGGGSGGGGSGGGGSQIVLTQSPAIMSASPGEKVTMTCSATSSVSYMHWYQQKSGTSPKRWIYDTSKLASGVPARFSGSGSGTSYSLTISSMEAEDAATYYCQQWSSNPLTFGAGTKLELK

SEQ ID NO: 9 - protein, 241 aa, Artificial Sequence
  BMA031.H6L12 scFv
QVQLVQSGAEVKKPGASVKVSCKASGYKFTSYVMHWVRQAPGQGLEWIGYINPYNDVTKYNEKFKGRVTITADKSTSTAYMELSSLRSEDTAVHYCARGSYYDYDGFVYWGQGTLVTVSSGGGGSGGGGSGGGGSEIVLTQSPATLSLSPGERATLSCSATSSVSYMHWYQQKPGKAPKRWIYDTSKLASGVPSRFSGSGSGTEFTLTISSLQPEDFATYYCQQWSSNPLTFGQGTKLEIK

SEQ ID NO: 10 - protein, 251 aa, Artificial Sequence
  αCD5.14 scFv
IDAMGNIQLVQSGPELKKPGETVKISCKASGYTFTNYGMNWVKQAPGKGLRWMGWINTHTGEPTYADDFKGRFAFSLETSASTAYLQINNLKNEDTATYFCTRRGYDWYFDVWGAGTTVTVSSGGGGSGGGGSGGGGSDIKMTQSPSSMYASLGERVTITCKASQDINSYLSWFHHKPGKSPKTLIYRANRLVDGVPSRFSGSGSGQDYSLTISSLDYEDMGIYYCQQYDESPWTFGGGTKLEMKGSGDPA

SEQ ID NO: 11 - protein, 244 aa, Artificial Sequence
  αCD7.TH69 scFv
EVQLVESGGGLVKPGGSLKLSCAASGLTFSSYAMSWVRQTPEKRLEWVASISSGGFTYYPDSVKGRFTISRDNARNILYLQMSSLRSEDTAMYYCARDEVRGYLDVWGAGTTVTVSSGGGGSGGGGSGGGGSAAYKDIQMTQTTSSLSASLGDRVTISCSASQGISNYLNWYQQKPDGTVKLLIYYTSSLHSGVPSRFSGSGSGTDYSLTISNLEPEDIATYYCQQYSKLPYTFGGGTKLEIKR

SEQ ID NO: 12 - protein, 244 aa, Artificial Sequence
  αPD-L1 scFv
EVQLVQSGGGVVQPGRSLRLSCAASGFTFSNYAMHWVRQAPGKGLEWVAIITYAGSNEYYADSVKGRFTISRDNSKNTLYLQMNSLRPEDTAVYYCARDRIWVDYWGQGTLVTVSSGGGGSGGGGSGGGGSDIQMTQSPDSLAVSLGERATINCKSSQSVLYSSNNKNYLAWYQQKPGQPPKLLIYWASTRESGVPDRFSGSGSGTDFTLTISSLQAEDVAVYYCQQYYSTPLTFGGGTKVEIK

SEQ ID NO: 13 - protein, 244 aa, Artificial Sequence
  αCD47 ScFv
QVQLVQSGAEVKKPGASVKVSCKASGYTFTNYNMHWVRQAPGQRLEWMGTIYPGNDDTSYNQKFKDRVTITADTSASTAYMELSSLRSEDTAVYYCARGGYRAMDYWGQGTLVTVSSGGGGSGGGGSGGGGSDIVMTQSPLSLPVTPGEPASISCRSSQSIVYSNGNTYLGWYLQKPGQSPQLLIYKVSNRFSGVPDRFSGSGSGTDFTLKISRVEAEDVGVYYCFQGSHVPYTFGQGTKLEIK

SEQ ID NO: 14 - protein, 23 aa, Artificial Sequence
  CD4 hinge
DSGQVLLESNIKVLPTWSTPVQP

SEQ ID NO: 15 - protein, 22 aa, Artificial Sequence
  CD4 Transmembrane domain
MALIVLGGVAGLLLFIGLGIFF

SEQ ID NO: 16 - protein, 46 aa, Artificial Sequence
  CD8α hinge
GTTTPAPRPPTPAPTIASQPLSLRPEACRPAAGGAVHTRGLDFACD

SEQ ID NO: 17 - protein, 24 aa, Artificial Sequence
  CD8α transmembrane domain(used in LS008*)
IYIWAPLAGTCGVLLLSLVITLYC

SEQ ID NO: 18 - protein, 21 aa, Artificial Sequence
  CD8α transmembrane domain
IYIWAPLAGTCGVLLLSLVIT

SEQ ID NO: 19 - protein, 21 aa, Artificial Sequence
  Signal Peptide (CD8α)
MALPVTALLLPLALLLHAARP

SEQ ID NO: 20 - protein, 19 aa, Artificial Sequence
  Signal Peptide(IGHV3-23)
MEFGLSWLFLVAILKGVQC

SEQ ID NO: 21 - protein, 303 aa, Artificial Sequence
  CHIP
MKGKEEKEGGARLGAGGGSPEKSPSAQELKEQGNRLFVGRKYPEAAACYGRAITRNPLVAVYYTNRALCYLKMQQHEQALADCRRALELDGQSVKAHFFLGQCQLEMESYDEAIANLQRAYSLAKEQRLNFGDDIPSALRIAKKKRWNSIEERRIHQESELHSYLSRLIAAERERELEECQRNHEGDEDDSHVRAQQACIEAKHDKYMADMDELFSQVDEKRKKRDIPDYLCGKISFELMREPCITPSGITYDRKDIEEHLQRVGHFDPVTRSPLTQEQLIPNLAMKEVIDAFISENGWVEDY

SEQ ID NO: 22 - protein, 176 aa, Artificial Sequence
  CHIP.dTPR(i.e.h CHIP.dTPR or hCHIP. ΔTPR)
RLNFGDDIPSALRIAKKKRWNSIEERRIHQESELHSYLSRLIAAERERELEECQRNHEGDEDDSHVRAQQACIEAKHDKYMADMDELFSQVDEKRKKRDIPDYLCGKISFELMREPCITPSGITYDRKDIEEHLQRVGHFDPVTRSPLTQEQLIPNLAMKEVIDAFISENGWVEDY

SEQ ID NO: 23 - protein, 292 aa, Artificial Sequence
  FBW7.2-293(i.e. FBW7)
CVPRSGLILSCICLYCGVLLPVLLPNLPFLTCLSMSTLESVTYLPEKGLYCQRLPSSRTHGGTESLKGKNTENMGFYGTLKMIFYKMKRKLDHGSEVRSFSLGKKPCKVSEYTSTTGLVPCSATPTTFGDLRAANGQGQQRRRITSVQPPTGLQEWLKMFQSWSGPEKLLALDELIDSCEPTQVKHMMQVIEPQFQRDFISLLPKELALYVLSFLEPKDLLQAAQTCRYWRILAEDNLLWREKCKEEGIDEPLHIKRRKVIKPGFIHSPWKSAYIRQHRIDTNWRRGELKSP

SEQ ID NO: 24 - protein, 62 aa, Artificial Sequence
  VHL.152-213(i.e.VHL)
TLPVYTLKERCLQVVRSLVKPENYRRLDIVRSLYEDLEDHPNVQKDLERLTQERIAHQRMGD

SEQ ID NO: 25 - protein, 208 aa, Artificial Sequence
  SPOP.167-374(i.e.SPOP)
SVNISGQNTMNMVKVPECRLADELGGLWENSRFTDCCLCVAGQEFQAHKAILAARSPVFSAMFEHEMEESKKNRVEINDVEPEVFKEMMCFIYTGKAPNLDKMADDLLAAADKYALERLKVMCEDALCSNLSVENAAEILILADLHSADQLKTQAVDFINYHASDVLETSGWKSMVVSHPHLVAEAYRSLASAQCPFLGPPRKRLKQS

SEQ ID NO: 26 - protein, 56 aa, Artificial Sequence
  SOCS2.143-198(i.e. SOCS2)
PRNGTVHLYLTKPLYTSAPSLQHLCRLTINKCTGAIWGLPLPTRLKDYLEEYKFQV

SEQ ID NO: 27 - protein, 486 aa, Artificial Sequence
  LS008*( αCD19 CAR)
MALPVTALLLPLALLLHAARPDIQMTQTTSSLSASLGDRVTISCRASQDISKYLNWYQQKPDGTVKLLIYHTSRLHSGVPSRFSGSGSGTDYSLTISNLEQEDIATYFCQQGNTLPYTFGGGTKLEITGGGGSGGGGSGGGGSEVKLQESGPGLVAPSQSLSVTCTVSGVSLPDYGVSWIRQPPRKGLEWLGVIWGSETTYYNSALKSRLTIIKDNSKSQVFLKMNSLQTDDTAIYYCAKHYYYGGSYAMDYWGQGTSVTVSSTTTPAPRPPTPAPTIASQPLSLRPEACRPAAGGAVHTRGLDFACDIYIWAPLAGTCGVLLLSLVITLYCKRGRKKLLYIFKQPFMRPVQTTQEEDGCSCRFPEEEEGGCELRVKFSRSADAPAYKQGQNQLYNELNLGRREEYDVLDKRRGRDPEMGGKPRRKNPQEGLYNELQKDKMAEAYSEIGMKGERRRGKGHDGLYQGLSTATKDTYDALHMQALPPR

SEQ ID NO: 28 - protein, 329 aa, Artificial Sequence
  LG024*
MALPVTALLLPLALLLHAARPQVQLVQSGGGVVQPGRSLRLSCKASGYTFTRYTMHWVRQAPGKGLEWIGYINPSRGYTNYNQKFKDRFTISRDNSKNTAFLQMDSLRPEDTGVYFCARYYDDHYSLDYWGQGTPVTVSSGGGGSGGGGSGGGGSDIQMTQSPSSLSASVGDRVTITCSASSSVSYMNWYQQTPGKAPKRWIYDTSKLASGVPSRFSGSGSGTDYTFTISSLQPEDIATYYCQQWSSNPFTFGQGTKLQITRGTTTPAPRPPTPAPTIASQPLSLRPEACRPAAGGAVHTRGLDFACDIYIWAPLAGTCGVLLLSLVIT

SEQ ID NO: 29 - protein, 424 aa, Artificial Sequence
  LG085*
QVQLVQSGGGVVQPGRSLRLSCKASGYTFTRYTMHWVRQAPGKGLEWIGYINPSRGYTNYNQKFKDRFTISRDNSKNTAFLQMDSLRPEDTGVYFCARYYDDHYSLDYWGQGTPVTVSSGGGGSGGGGSGGGGSDIQMTQSPSSLSASVGDRVTITCSASSSVSYMNWYQQTPGKAPKRWIYDTSKLASGVPSRFSGSGSGTDYTFTISSLQPEDIATYYCQQWSSNPFTFGQGTKLQITRGSGSGSGRLNFGDDIPSALRIAKKKRWNSIEERRIHQESELHSYLSRLIAAERERELEECQRNHEGDEDDSHVRAQQACIEAKHDKYMADMDELFSQVDEKRKKRDIPDYLCGKISFELMREPCITPSGITYDRKDIEEHLQRVGHFDPVTRSPLTQEQLIPNLAMKEVIDAFISENGWVEDY

SEQ ID NO: 30 - protein, 553 aa, Artificial Sequence
  LG089*
CVPRSGLILSCICLYCGVLLPVLLPNLPFLTCLSMSTLESVTYLPEKGLYCQRLPSSRTHGGTESLKGKNTENMGFYGTLKMIFYKMKRKLDHGSEVRSFSLGKKPCKVSEYTSTTGLVPCSATPTTFGDLRAANGQGQQRRRITSVQPPTGLQEWLKMFQSWSGPEKLLALDELIDSCEPTQVKHMMQVIEPQFQRDFISLLPKELALYVLSFLEPKDLLQAAQTCRYWRILAEDNLLWREKCKEEGIDEPLHIKRRKVIKPGFIHSPWKSAYIRQHRIDTNWRRGELKSPGSGSGSGEVQLVESGGGLVQPGGSLKLSCAASGFTFNKYAMNWVRQAPGKGLEWVARIRSKYNNYATYYADSVKDRFTISRDDSKNTAYLQMNNLKTEDTAVYYCVRHGNFGNSYISYWAYWGQGTLVTVSSGGGGSGGGGSGGGGSGGGGSQTVVTQEPSLTVSPGGTVTLTCGSSTGAVTSGYYPNWVQQKPGQAPRGLIGGTKFLAPGTPARFSGSLLGGKAALTLSGVQPEDEAEYYCALWYSNRWVFGGGTKLTVL

SEQ ID NO: 31 - protein, 323 aa, Artificial Sequence
  LG091*
EVQLVESGGGLVQPGGSLKLSCAASGFTFNKYAMNWVRQAPGKGLEWVARIRSKYNNYATYYADSVKDRFTISRDDSKNTAYLQMNNLKTEDTAVYYCVRHGNFGNSYISYWAYWGQGTLVTVSSGGGGSGGGGSGGGGSGGGGSQTVVTQEPSLTVSPGGTVTLTCGSSTGAVTSGYYPNWVQQKPGQAPRGLIGGTKFLAPGTPARFSGSLLGGKAALTLSGVQPEDEAEYYCALWYSNRWVFGGGTKLTVLGSGSGSGTLPVYTLKERCLQVVRSLVKPENYRRLDIVRSLYEDLEDHPNVQKDLERLTQERIAHQRMGD

SEQ ID NO: 32 - protein, 469 aa, Artificial Sequence
  LG092*
EVQLVESGGGLVQPGGSLKLSCAASGFTFNKYAMNWVRQAPGKGLEWVARIRSKYNNYATYYADSVKDRFTISRDDSKNTAYLQMNNLKTEDTAVYYCVRHGNFGNSYISYWAYWGQGTLVTVSSGGGGSGGGGSGGGGSGGGGSQTVVTQEPSLTVSPGGTVTLTCGSSTGAVTSGYYPNWVQQKPGQAPRGLIGGTKFLAPGTPARFSGSLLGGKAALTLSGVQPEDEAEYYCALWYSNRWVFGGGTKLTVLGSGSGSGSVNISGQNTMNMVKVPECRLADELGGLWENSRFTDCCLCVAGQEFQAHKAILAARSPVFSAMFEHEMEESKKNRVEINDVEPEVFKEMMCFIYTGKAPNLDKMADDLLAAADKYALERLKVMCEDALCSNLSVENAAEILILADLHSADQLKTQAVDFINYHASDVLETSGWKSMVVSHPHLVAEAYRSLASAQCPFLGPPRKRLKQS

SEQ ID NO: 33 - protein, 512 aa, Artificial Sequence
  LG112*
MALPVTALLLPLALLLHAARPQVQLVQSGGGVVQPGRSLRLSCKASGYTFTRYTMHWVRQAPGKGLEWIGYINPSRGYTNYNQKFKDRFTISRDNSKNTAFLQMDSLRPEDTGVYFCARYYDDHYSLDYWGQGTPVTVSSGGGGSGGGGSGGGGSDIQMTQSPSSLSASVGDRVTITCSASSSVSYMNWYQQTPGKAPKRWIYDTSKLASGVPSRFSGSGSGTDYTFTISSLQPEDIATYYCQQWSSNPFTFGQGTKLQITRGSGSGSGRLNFGDDIPSALRIAKKKRWNSIEERRIHQESELHSYLSRLIAAERERELEECQRNHEGDEDDSHVRAQQACIEAKHDKYMADMDELFSQVDEKRKKRDIPDYLCGKISFELMREPCITPSGITYDRKDIEEHLQRVGHFDPVTRSPLTQEQLIPNLAMKEVIDAFISENGWVEDYGTTTPAPRPPTPAPTIASQPLSLRPEACRPAAGGAVHTRGLDFACDIYIWAPLAGTCGVLLLSLVIT

SEQ ID NO: 34 - protein, 491 aa, Artificial Sequence
  LG112*△SP
QVQLVQSGGGVVQPGRSLRLSCKASGYTFTRYTMHWVRQAPGKGLEWIGYINPSRGYTNYNQKFKDRFTISRDNSKNTAFLQMDSLRPEDTGVYFCARYYDDHYSLDYWGQGTPVTVSSGGGGSGGGGSGGGGSDIQMTQSPSSLSASVGDRVTITCSASSSVSYMNWYQQTPGKAPKRWIYDTSKLASGVPSRFSGSGSGTDYTFTISSLQPEDIATYYCQQWSSNPFTFGQGTKLQITRGSGSGSGRLNFGDDIPSALRIAKKKRWNSIEERRIHQESELHSYLSRLIAAERERELEECQRNHEGDEDDSHVRAQQACIEAKHDKYMADMDELFSQVDEKRKKRDIPDYLCGKISFELMREPCITPSGITYDRKDIEEHLQRVGHFDPVTRSPLTQEQLIPNLAMKEVIDAFISENGWVEDYGTTTPAPRPPTPAPTIASQPLSLRPEACRPAAGGAVHTRGLDFACDIYIWAPLAGTCGVLLLSLVIT

SEQ ID NO: 35 - protein, 512 aa, Artificial Sequence
  LG113*
MALPVTALLLPLALLLHAARPQVQLVQSGGGVVQPGRSLRLSCKASGYTFTRYTMHWVRQAPGKGLEWIGYINPSRGYTNYNQKFKDRFTISRDNSKNTAFLQMDSLRPEDTGVYFCARYYDDHYSLDYWGQGTPVTVSSGGGGSGGGGSGGGGSDIQMTQSPSSLSASVGDRVTITCSASSSVSYMNWYQQTPGKAPKRWIYDTSKLASGVPSRFSGSGSGTDYTFTISSLQPEDIATYYCQQWSSNPFTFGQGTKLQITRGTTTPAPRPPTPAPTIASQPLSLRPEACRPAAGGAVHTRGLDFACDIYIWAPLAGTCGVLLLSLVITGSGSGSGRLNFGDDIPSALRIAKKKRWNSIEERRIHQESELHSYLSRLIAAERERELEECQRNHEGDEDDSHVRAQQACIEAKHDKYMADMDELFSQVDEKRKKRDIPDYLCGKISFELMREPCITPSGITYDRKDIEEHLQRVGHFDPVTRSPLTQEQLIPNLAMKEVIDAFISENGWVEDY

SEQ ID NO: 36 - protein, 491 aa, Artificial Sequence
  LG113*△SP
QVQLVQSGGGVVQPGRSLRLSCKASGYTFTRYTMHWVRQAPGKGLEWIGYINPSRGYTNYNQKFKDRFTISRDNSKNTAFLQMDSLRPEDTGVYFCARYYDDHYSLDYWGQGTPVTVSSGGGGSGGGGSGGGGSDIQMTQSPSSLSASVGDRVTITCSASSSVSYMNWYQQTPGKAPKRWIYDTSKLASGVPSRFSGSGSGTDYTFTISSLQPEDIATYYCQQWSSNPFTFGQGTKLQITRGTTTPAPRPPTPAPTIASQPLSLRPEACRPAAGGAVHTRGLDFACDIYIWAPLAGTCGVLLLSLVITGSGSGSGRLNFGDDIPSALRIAKKKRWNSIEERRIHQESELHSYLSRLIAAERERELEECQRNHEGDEDDSHVRAQQACIEAKHDKYMADMDELFSQVDEKRKKRDIPDYLCGKISFELMREPCITPSGITYDRKDIEEHLQRVGHFDPVTRSPLTQEQLIPNLAMKEVIDAFISENGWVEDY

SEQ ID NO: 37 - protein, 521 aa, Artificial Sequence
  LG123*
MALPVTALLLPLALLLHAARPMDIQMTQTTSSLSASLGDRVTISCRASQDIRNYLNWYQQKPDGTVKLLIYYTSRLHSGVPSKFSGSGSGTDYSLTISNLEQEDIATYFCQQGNTLPWTFAGGTKLEIKGGGGSGGGGSGGGGSGGGGSEVQLQQSGPELVKPGASMKISCKASGYSFTGYTMNWVKQSHGKNLEWMGLINPYKGVSTYNQKFKDKATLTVDKSSSTAYMELLSLTSEDSAVYYCARSGYYGDSDWYFDVWGQGTTLTVFSGSGSGSGRLNFGDDIPSALRIAKKKRWNSIEERRIHQESELHSYLSRLIAAERERELEECQRNHEGDEDDSHVRAQQACIEAKHDKYMADMDELFSQVDEKRKKRDIPDYLCGKISFELMREPCITPSGITYDRKDIEEHLQRVGHFDPVTRSPLTQEQLIPNLAMKEVIDAFISENGWVEDYGTTTPAPRPPTPAPTIASQPLSLRPEACRPAAGGAVHTRGLDFACDIYIWAPLAGTCGVLLLSLVIT

SEQ ID NO: 38 - protein, 500 aa, Artificial Sequence
  LG123*△SP
MDIQMTQTTSSLSASLGDRVTISCRASQDIRNYLNWYQQKPDGTVKLLIYYTSRLHSGVPSKFSGSGSGTDYSLTISNLEQEDIATYFCQQGNTLPWTFAGGTKLEIKGGGGSGGGGSGGGGSGGGGSEVQLQQSGPELVKPGASMKISCKASGYSFTGYTMNWVKQSHGKNLEWMGLINPYKGVSTYNQKFKDKATLTVDKSSSTAYMELLSLTSEDSAVYYCARSGYYGDSDWYFDVWGQGTTLTVFSGSGSGSGRLNFGDDIPSALRIAKKKRWNSIEERRIHQESELHSYLSRLIAAERERELEECQRNHEGDEDDSHVRAQQACIEAKHDKYMADMDELFSQVDEKRKKRDIPDYLCGKISFELMREPCITPSGITYDRKDIEEHLQRVGHFDPVTRSPLTQEQLIPNLAMKEVIDAFISENGWVEDYGTTTPAPRPPTPAPTIASQPLSLRPEACRPAAGGAVHTRGLDFACDIYIWAPLAGTCGVLLLSLVIT

SEQ ID NO: 39 - protein, 516 aa, Artificial Sequence
  LG124*
MALPVTALLLPLALLLHAARPMDIQMTQSPSSLSASVGDRVTITCRASQDIRNYLNWYQQKPGKAPKLLIYYTSRLESGVPSRFSGSGSGTDYTLTISSLQPEDFATYYCQQGNTLPWTFGQGTKVEIKGGGGSGGGGSGGGGSEVQLVESGGGLVQPGGSLRLSCAASGYSFTGYTMNWVRQAPGKGLEWVALINPTKGVSTYNQKFKDRFTISVDKSKNTAYLQMNSLRAEDTAVYYCARSGYYGDSDWYFDVWGQGTLVTVSSGSGSGSGRLNFGDDIPSALRIAKKKRWNSIEERRIHQESELHSYLSRLIAAERERELEECQRNHEGDEDDSHVRAQQACIEAKHDKYMADMDELFSQVDEKRKKRDIPDYLCGKISFELMREPCITPSGITYDRKDIEEHLQRVGHFDPVTRSPLTQEQLIPNLAMKEVIDAFISENGWVEDYGTTTPAPRPPTPAPTIASQPLSLRPEACRPAAGGAVHTRGLDFACDIYIWAPLAGTCGVLLLSLVIT

SEQ ID NO: 40 - protein, 495 aa, Artificial Sequence
  LG124*△SP
MDIQMTQSPSSLSASVGDRVTITCRASQDIRNYLNWYQQKPGKAPKLLIYYTSRLESGVPSRFSGSGSGTDYTLTISSLQPEDFATYYCQQGNTLPWTFGQGTKVEIKGGGGSGGGGSGGGGSEVQLVESGGGLVQPGGSLRLSCAASGYSFTGYTMNWVRQAPGKGLEWVALINPTKGVSTYNQKFKDRFTISVDKSKNTAYLQMNSLRAEDTAVYYCARSGYYGDSDWYFDVWGQGTLVTVSSGSGSGSGRLNFGDDIPSALRIAKKKRWNSIEERRIHQESELHSYLSRLIAAERERELEECQRNHEGDEDDSHVRAQQACIEAKHDKYMADMDELFSQVDEKRKKRDIPDYLCGKISFELMREPCITPSGITYDRKDIEEHLQRVGHFDPVTRSPLTQEQLIPNLAMKEVIDAFISENGWVEDYGTTTPAPRPPTPAPTIASQPLSLRPEACRPAAGGAVHTRGLDFACDIYIWAPLAGTCGVLLLSLVIT

SEQ ID NO: 41 - protein, 511 aa, Artificial Sequence
  LG125*
MALPVTALLLPLALLLHAARPDIQLTQSPAIMSASPGEKVTMTCRASSSVSYMNWYQQKSGTSPKRWIYDTSKVASGVPYRFSGSGSGTSYSLTISSMEAEDAATYYCQQWSSNPLTFGAGTKLELKGGGGSGGGGSGGGGSDIKLQQSGAELARPGASVKMSCKTSGYTFTRYTMHWVKQRPGQGLEWIGYINPSRGYTNYNQKFKDKATLTTDKSSSTAYMQLSSLTSEDSAVYYCARYYDDHYCLDYWGQGTTLTVSSGSGSGSGRLNFGDDIPSALRIAKKKRWNSIEERRIHQESELHSYLSRLIAAERERELEECQRNHEGDEDDSHVRAQQACIEAKHDKYMADMDELFSQVDEKRKKRDIPDYLCGKISFELMREPCITPSGITYDRKDIEEHLQRVGHFDPVTRSPLTQEQLIPNLAMKEVIDAFISENGWVEDYGTTTPAPRPPTPAPTIASQPLSLRPEACRPAAGGAVHTRGLDFACDIYIWAPLAGTCGVLLLSLVIT

SEQ ID NO: 42 - protein, 490 aa, Artificial Sequence
  LG125*△SP
DIQLTQSPAIMSASPGEKVTMTCRASSSVSYMNWYQQKSGTSPKRWIYDTSKVASGVPYRFSGSGSGTSYSLTISSMEAEDAATYYCQQWSSNPLTFGAGTKLELKGGGGSGGGGSGGGGSDIKLQQSGAELARPGASVKMSCKTSGYTFTRYTMHWVKQRPGQGLEWIGYINPSRGYTNYNQKFKDKATLTTDKSSSTAYMQLSSLTSEDSAVYYCARYYDDHYCLDYWGQGTTLTVSSGSGSGSGRLNFGDDIPSALRIAKKKRWNSIEERRIHQESELHSYLSRLIAAERERELEECQRNHEGDEDDSHVRAQQACIEAKHDKYMADMDELFSQVDEKRKKRDIPDYLCGKISFELMREPCITPSGITYDRKDIEEHLQRVGHFDPVTRSPLTQEQLIPNLAMKEVIDAFISENGWVEDYGTTTPAPRPPTPAPTIASQPLSLRPEACRPAAGGAVHTRGLDFACDIYIWAPLAGTCGVLLLSLVIT

SEQ ID NO: 43 - protein, 520 aa, Artificial Sequence
  LG126*
MALPVTALLLPLALLLHAARPQTVVTQEPSLTVSPGGTVTLTCGSSTGAVTSGYYPNWVQQKPGQAPRGLIGGTKFLAPGTPARFSGSLLGGKAALTLSGVQPEDEAEYYCALWYSNRWVFGGGTKLTVLGGGGSGGGGSGGGGSEVQLLESGGGLVQPGGSLKLSCAASGFTFNIYAMNWVRQAPGKGLEWVARIRSKYNNYATYYADSVKSRFTISRDDSKNTAYLQMNNLKTEDTAVYYCVRHGNFGNSYVSFFAYWGQGTLVTVSSGSGSGSGRLNFGDDIPSALRIAKKKRWNSIEERRIHQESELHSYLSRLIAAERERELEECQRNHEGDEDDSHVRAQQACIEAKHDKYMADMDELFSQVDEKRKKRDIPDYLCGKISFELMREPCITPSGITYDRKDIEEHLQRVGHFDPVTRSPLTQEQLIPNLAMKEVIDAFISENGWVEDYGTTTPAPRPPTPAPTIASQPLSLRPEACRPAAGGAVHTRGLDFACDIYIWAPLAGTCGVLLLSLVIT

SEQ ID NO: 44 - protein, 499 aa, Artificial Sequence
  LG126*△SP
QTVVTQEPSLTVSPGGTVTLTCGSSTGAVTSGYYPNWVQQKPGQAPRGLIGGTKFLAPGTPARFSGSLLGGKAALTLSGVQPEDEAEYYCALWYSNRWVFGGGTKLTVLGGGGSGGGGSGGGGSEVQLLESGGGLVQPGGSLKLSCAASGFTFNIYAMNWVRQAPGKGLEWVARIRSKYNNYATYYADSVKSRFTISRDDSKNTAYLQMNNLKTEDTAVYYCVRHGNFGNSYVSFFAYWGQGTLVTVSSGSGSGSGRLNFGDDIPSALRIAKKKRWNSIEERRIHQESELHSYLSRLIAAERERELEECQRNHEGDEDDSHVRAQQACIEAKHDKYMADMDELFSQVDEKRKKRDIPDYLCGKISFELMREPCITPSGITYDRKDIEEHLQRVGHFDPVTRSPLTQEQLIPNLAMKEVIDAFISENGWVEDYGTTTPAPRPPTPAPTIASQPLSLRPEACRPAAGGAVHTRGLDFACDIYIWAPLAGTCGVLLLSLVIT

SEQ ID NO: 45 - protein, 512 aa, Artificial Sequence
  LG119*
MALPVTALLLPLALLLHAARPEVQLQQSGPELVKPGASVKMSCKASGYKFTSYVMHWVKQKPGQGLEWIGYINPYNDVTKYNEKFKGKATLTSDKSSSTAYMELSSLTSEDSAVHYCARGSYYDYDGFVYWGQGTLVTVSAGGGGSGGGGSGGGGSQIVLTQSPAIMSASPGEKVTMTCSATSSVSYMHWYQQKSGTSPKRWIYDTSKLASGVPARFSGSGSGTSYSLTISSMEAEDAATYYCQQWSSNPLTFGAGTKLELKGSGSGSGRLNFGDDIPSALRIAKKKRWNSIEERRIHQESELHSYLSRLIAAERERELEECQRNHEGDEDDSHVRAQQACIEAKHDKYMADMDELFSQVDEKRKKRDIPDYLCGKISFELMREPCITPSGITYDRKDIEEHLQRVGHFDPVTRSPLTQEQLIPNLAMKEVIDAFISENGWVEDYGTTTPAPRPPTPAPTIASQPLSLRPEACRPAAGGAVHTRGLDFACDIYIWAPLAGTCGVLLLSLVIT

SEQ ID NO: 46 - protein, 491 aa, Artificial Sequence
  LG119*△SP
EVQLQQSGPELVKPGASVKMSCKASGYKFTSYVMHWVKQKPGQGLEWIGYINPYNDVTKYNEKFKGKATLTSDKSSSTAYMELSSLTSEDSAVHYCARGSYYDYDGFVYWGQGTLVTVSAGGGGSGGGGSGGGGSQIVLTQSPAIMSASPGEKVTMTCSATSSVSYMHWYQQKSGTSPKRWIYDTSKLASGVPARFSGSGSGTSYSLTISSMEAEDAATYYCQQWSSNPLTFGAGTKLELKGSGSGSGRLNFGDDIPSALRIAKKKRWNSIEERRIHQESELHSYLSRLIAAERERELEECQRNHEGDEDDSHVRAQQACIEAKHDKYMADMDELFSQVDEKRKKRDIPDYLCGKISFELMREPCITPSGITYDRKDIEEHLQRVGHFDPVTRSPLTQEQLIPNLAMKEVIDAFISENGWVEDYGTTTPAPRPPTPAPTIASQPLSLRPEACRPAAGGAVHTRGLDFACDIYIWAPLAGTCGVLLLSLVIT

SEQ ID NO: 47 - protein, 512 aa, Artificial Sequence
  LG120*
MALPVTALLLPLALLLHAARPQVQLVQSGAEVKKPGASVKVSCKASGYKFTSYVMHWVRQAPGQGLEWIGYINPYNDVTKYNEKFKGRVTITADKSTSTAYMELSSLRSEDTAVHYCARGSYYDYDGFVYWGQGTLVTVSSGGGGSGGGGSGGGGSEIVLTQSPATLSLSPGERATLSCSATSSVSYMHWYQQKPGKAPKRWIYDTSKLASGVPSRFSGSGSGTEFTLTISSLQPEDFATYYCQQWSSNPLTFGQGTKLEIKGSGSGSGRLNFGDDIPSALRIAKKKRWNSIEERRIHQESELHSYLSRLIAAERERELEECQRNHEGDEDDSHVRAQQACIEAKHDKYMADMDELFSQVDEKRKKRDIPDYLCGKISFELMREPCITPSGITYDRKDIEEHLQRVGHFDPVTRSPLTQEQLIPNLAMKEVIDAFISENGWVEDYGTTTPAPRPPTPAPTIASQPLSLRPEACRPAAGGAVHTRGLDFACDIYIWAPLAGTCGVLLLSLVIT

SEQ ID NO: 48 - protein, 491 aa, Artificial Sequence
  LG120*△SP
QVQLVQSGAEVKKPGASVKVSCKASGYKFTSYVMHWVRQAPGQGLEWIGYINPYNDVTKYNEKFKGRVTITADKSTSTAYMELSSLRSEDTAVHYCARGSYYDYDGFVYWGQGTLVTVSSGGGGSGGGGSGGGGSEIVLTQSPATLSLSPGERATLSCSATSSVSYMHWYQQKPGKAPKRWIYDTSKLASGVPSRFSGSGSGTEFTLTISSLQPEDFATYYCQQWSSNPLTFGQGTKLEIKGSGSGSGRLNFGDDIPSALRIAKKKRWNSIEERRIHQESELHSYLSRLIAAERERELEECQRNHEGDEDDSHVRAQQACIEAKHDKYMADMDELFSQVDEKRKKRDIPDYLCGKISFELMREPCITPSGITYDRKDIEEHLQRVGHFDPVTRSPLTQEQLIPNLAMKEVIDAFISENGWVEDYGTTTPAPRPPTPAPTIASQPLSLRPEACRPAAGGAVHTRGLDFACDIYIWAPLAGTCGVLLLSLVIT

SEQ ID NO: 49 - protein, 520 aa, Artificial Sequence
  LG137*
MEFGLSWLFLVAILKGVQCIDAMGNIQLVQSGPELKKPGETVKISCKASGYTFTNYGMNWVKQAPGKGLRWMGWINTHTGEPTYADDFKGRFAFSLETSASTAYLQINNLKNEDTATYFCTRRGYDWYFDVWGAGTTVTVSSGGGGSGGGGSGGGGSDIKMTQSPSSMYASLGERVTITCKASQDINSYLSWFHHKPGKSPKTLIYRANRLVDGVPSRFSGSGSGQDYSLTISSLDYEDMGIYYCQQYDESPWTFGGGTKLEMKGSGDPAGSGSGSGRLNFGDDIPSALRIAKKKRWNSIEERRIHQESELHSYLSRLIAAERERELEECQRNHEGDEDDSHVRAQQACIEAKHDKYMADMDELFSQVDEKRKKRDIPDYLCGKISFELMREPCITPSGITYDRKDIEEHLQRVGHFDPVTRSPLTQEQLIPNLAMKEVIDAFISENGWVEDYGTTTPAPRPPTPAPTIASQPLSLRPEACRPAAGGAVHTRGLDFACDIYIWAPLAGTCGVLLLSLVIT

SEQ ID NO: 50 - protein, 500 aa, Artificial Sequence
  LG137*△SP
DAMGNIQLVQSGPELKKPGETVKISCKASGYTFTNYGMNWVKQAPGKGLRWMGWINTHTGEPTYADDFKGRFAFSLETSASTAYLQINNLKNEDTATYFCTRRGYDWYFDVWGAGTTVTVSSGGGGSGGGGSGGGGSDIKMTQSPSSMYASLGERVTITCKASQDINSYLSWFHHKPGKSPKTLIYRANRLVDGVPSRFSGSGSGQDYSLTISSLDYEDMGIYYCQQYDESPWTFGGGTKLEMKGSGDPAGSGSGSGRLNFGDDIPSALRIAKKKRWNSIEERRIHQESELHSYLSRLIAAERERELEECQRNHEGDEDDSHVRAQQACIEAKHDKYMADMDELFSQVDEKRKKRDIPDYLCGKISFELMREPCITPSGITYDRKDIEEHLQRVGHFDPVTRSPLTQEQLIPNLAMKEVIDAFISENGWVEDYGTTTPAPRPPTPAPTIASQPLSLRPEACRPAAGGAVHTRGLDFACDIYIWAPLAGTCGVLLLSLVIT

SEQ ID NO: 51 - protein, 515 aa, Artificial Sequence
  LG138*
MALPVTALLLPLALLLHAARPEVQLVESGGGLVKPGGSLKLSCAASGLTFSSYAMSWVRQTPEKRLEWVASISSGGFTYYPDSVKGRFTISRDNARNILYLQMSSLRSEDTAMYYCARDEVRGYLDVWGAGTTVTVSSGGGGSGGGGSGGGGSAAYKDIQMTQTTSSLSASLGDRVTISCSASQGISNYLNWYQQKPDGTVKLLIYYTSSLHSGVPSRFSGSGSGTDYSLTISNLEPEDIATYYCQQYSKLPYTFGGGTKLEIKRGSGSGSGRLNFGDDIPSALRIAKKKRWNSIEERRIHQESELHSYLSRLIAAERERELEECQRNHEGDEDDSHVRAQQACIEAKHDKYMADMDELFSQVDEKRKKRDIPDYLCGKISFELMREPCITPSGITYDRKDIEEHLQRVGHFDPVTRSPLTQEQLIPNLAMKEVIDAFISENGWVEDYGTTTPAPRPPTPAPTIASQPLSLRPEACRPAAGGAVHTRGLDFACDIYIWAPLAGTCGVLLLSLVIT

SEQ ID NO: 52 - protein, 494 aa, Artificial Sequence
  LG138*△SP
EVQLVESGGGLVKPGGSLKLSCAASGLTFSSYAMSWVRQTPEKRLEWVASISSGGFTYYPDSVKGRFTISRDNARNILYLQMSSLRSEDTAMYYCARDEVRGYLDVWGAGTTVTVSSGGGGSGGGGSGGGGSAAYKDIQMTQTTSSLSASLGDRVTISCSASQGISNYLNWYQQKPDGTVKLLIYYTSSLHSGVPSRFSGSGSGTDYSLTISNLEPEDIATYYCQQYSKLPYTFGGGTKLEIKRGSGSGSGRLNFGDDIPSALRIAKKKRWNSIEERRIHQESELHSYLSRLIAAERERELEECQRNHEGDEDDSHVRAQQACIEAKHDKYMADMDELFSQVDEKRKKRDIPDYLCGKISFELMREPCITPSGITYDRKDIEEHLQRVGHFDPVTRSPLTQEQLIPNLAMKEVIDAFISENGWVEDYGTTTPAPRPPTPAPTIASQPLSLRPEACRPAAGGAVHTRGLDFACDIYIWAPLAGTCGVLLLSLVIT

SEQ ID NO: 53 - protein, 515 aa, Artificial Sequence
  MLB052*
MALPVTALLLPLALLLHAARPEVQLVQSGGGVVQPGRSLRLSCAASGFTFSNYAMHWVRQAPGKGLEWVAIITYAGSNEYYADSVKGRFTISRDNSKNTLYLQMNSLRPEDTAVYYCARDRIWVDYWGQGTLVTVSSGGGGSGGGGSGGGGSDIQMTQSPDSLAVSLGERATINCKSSQSVLYSSNNKNYLAWYQQKPGQPPKLLIYWASTRESGVPDRFSGSGSGTDFTLTISSLQAEDVAVYYCQQYYSTPLTFGGGTKVEIKGSGSGSGRLNFGDDIPSALRIAKKKRWNSIEERRIHQESELHSYLSRLIAAERERELEECQRNHEGDEDDSHVRAQQACIEAKHDKYMADMDELFSQVDEKRKKRDIPDYLCGKISFELMREPCITPSGITYDRKDIEEHLQRVGHFDPVTRSPLTQEQLIPNLAMKEVIDAFISENGWVEDYGTTTPAPRPPTPAPTIASQPLSLRPEACRPAAGGAVHTRGLDFACDIYIWAPLAGTCGVLLLSLVIT

SEQ ID NO: 54 - protein, 494 aa, Artificial Sequence
  MLB052*△SP
EVQLVQSGGGVVQPGRSLRLSCAASGFTFSNYAMHWVRQAPGKGLEWVAIITYAGSNEYYADSVKGRFTISRDNSKNTLYLQMNSLRPEDTAVYYCARDRIWVDYWGQGTLVTVSSGGGGSGGGGSGGGGSDIQMTQSPDSLAVSLGERATINCKSSQSVLYSSNNKNYLAWYQQKPGQPPKLLIYWASTRESGVPDRFSGSGSGTDFTLTISSLQAEDVAVYYCQQYYSTPLTFGGGTKVEIKGSGSGSGRLNFGDDIPSALRIAKKKRWNSIEERRIHQESELHSYLSRLIAAERERELEECQRNHEGDEDDSHVRAQQACIEAKHDKYMADMDELFSQVDEKRKKRDIPDYLCGKISFELMREPCITPSGITYDRKDIEEHLQRVGHFDPVTRSPLTQEQLIPNLAMKEVIDAFISENGWVEDYGTTTPAPRPPTPAPTIASQPLSLRPEACRPAAGGAVHTRGLDFACDIYIWAPLAGTCGVLLLSLVIT

SEQ ID NO: 55 - protein, 515 aa, Artificial Sequence
  MLB053*
MALPVTALLLPLALLLHAARPQVQLVQSGAEVKKPGASVKVSCKASGYTFTNYNMHWVRQAPGQRLEWMGTIYPGNDDTSYNQKFKDRVTITADTSASTAYMELSSLRSEDTAVYYCARGGYRAMDYWGQGTLVTVSSGGGGSGGGGSGGGGSDIVMTQSPLSLPVTPGEPASISCRSSQSIVYSNGNTYLGWYLQKPGQSPQLLIYKVSNRFSGVPDRFSGSGSGTDFTLKISRVEAEDVGVYYCFQGSHVPYTFGQGTKLEIKGSGSGSGRLNFGDDIPSALRIAKKKRWNSIEERRIHQESELHSYLSRLIAAERERELEECQRNHEGDEDDSHVRAQQACIEAKHDKYMADMDELFSQVDEKRKKRDIPDYLCGKISFELMREPCITPSGITYDRKDIEEHLQRVGHFDPVTRSPLTQEQLIPNLAMKEVIDAFISENGWVEDYGTTTPAPRPPTPAPTIASQPLSLRPEACRPAAGGAVHTRGLDFACDIYIWAPLAGTCGVLLLSLVIT

SEQ ID NO: 56 - protein, 494 aa, Artificial Sequence
  MLB053*△SP
QVQLVQSGAEVKKPGASVKVSCKASGYTFTNYNMHWVRQAPGQRLEWMGTIYPGNDDTSYNQKFKDRVTITADTSASTAYMELSSLRSEDTAVYYCARGGYRAMDYWGQGTLVTVSSGGGGSGGGGSGGGGSDIVMTQSPLSLPVTPGEPASISCRSSQSIVYSNGNTYLGWYLQKPGQSPQLLIYKVSNRFSGVPDRFSGSGSGTDFTLKISRVEAEDVGVYYCFQGSHVPYTFGQGTKLEIKGSGSGSGRLNFGDDIPSALRIAKKKRWNSIEERRIHQESELHSYLSRLIAAERERELEECQRNHEGDEDDSHVRAQQACIEAKHDKYMADMDELFSQVDEKRKKRDIPDYLCGKISFELMREPCITPSGITYDRKDIEEHLQRVGHFDPVTRSPLTQEQLIPNLAMKEVIDAFISENGWVEDYGTTTPAPRPPTPAPTIASQPLSLRPEACRPAAGGAVHTRGLDFACDIYIWAPLAGTCGVLLLSLVIT

SEQ ID NO: 57 - protein, 258 aa, Artificial Sequence
  P2A-GFP**(i.e. P2A-eGFP)
ATNFSLLKQAGDVEENPGPMVSKGEELFTGVVPILVELDGDVNGHKFSVSGEGEGDATYGKLTLKFICTTGKLPVPWPTLVTTLTYGVQCFSRYPDHMKQHDFFKSAMPEGYVQERTIFFKDDGNYKTRAEVKFEGDTLVNRIELKGIDFKEDGNILGHKLEYNYNSHNVYIMADKQKNGIKVNFKIRHNIEDGSVQLADHYQQNTPIGDGPVLLPDNHYLSTQSALSKDPNEKRDHMVLLEFVTAAGITLGMDELYK

SEQ ID NO: 58 - protein, 27 aa, Artificial Sequence
  IL2Rβjm(i.e. IL2Rβ jm DT or L2Rβ jm domain)
NCRNTGPWLKKVLKCNTPDPSKFFSQL

SEQ ID NO: 59 - protein, 78 aa, Artificial Sequence
  MLB014*(CD3ζ.△IC-IL2Rβjm)
MKWKALFTAAILQAQLPITEAQSFGLLDPKLCYLLDGILFIYGVILTALFLNCRNTGPWLKKVLKCNTPDPSKFFSQL

SEQ ID NO: 60 - protein, 179 aa, Artificial Sequence
  MLB046 *(CD3ε.△IC -IL2Rβjm)
MQSGTHWRVLGLCLLSVGVWGQDGNEEMGGITQTPYKVSISGTTVILTCPQYPGSEILWQHNDKNIGGDEDDKNIGSDEDHLSLKEFSELEQSGYYVCYPRGSKPEDANFYLYLRARVCENCMEMDVMSVATIVIVDICITGGLLLLVYYWSNCRNTGPWLKKVLKCNTPDPSKFFSQL

SEQ ID NO: 61 - protein, 51 aa, Artificial Sequence
  CD3ζ.△IC
MKWKALFTAAILQAQLPITEAQSFGLLDPKLCYLLDGILFIYGVILTALFL

SEQ ID NO: 62 - protein, 200 aa, Artificial Sequence
  GRAIL.IC
YSARRLRNARAQSRKQRQLKADAKKAIGRLQLRTLKQGDKEIGPDGDSCAVCIELYKPNDLVRILTCNHIFHKTCVDPWLLEHRTCPMCKCDILKALGIEVDVEDGSVSLQVPVSNEISNSASSHEEDNRSETASSGYASVQGTDEPPLEEHVQSTNESLQLVNHEANSVAVDVIPHVDNPTFEEDETPNQETAVREIKS

SEQ ID NO: 63 - protein, 251 aa, Artificial Sequence
  LG171 *(CD3ζ.△IC-GRAIL.IC)
MKWKALFTAAILQAQLPITEAQSFGLLDPKLCYLLDGILFIYGVILTALFLYSARRLRNARAQSRKQRQLKADAKKAIGRLQLRTLKQGDKEIGPDGDSCAVCIELYKPNDLVRILTCNHIFHKTCVDPWLLEHRTCPMCKCDILKALGIEVDVEDGSVSLQVPVSNEISNSASSHEEDNRSETASSGYASVQGTDEPPLEEHVQSTNESLQLVNHEANSVAVDVIPHVDNPTFEEDETPNQETAVREIKS

SEQ ID NO: 64 - protein, 152 aa, Artificial Sequence
  CD3ε.△IC
MQSGTHWRVLGLCLLSVGVWGQDGNEEMGGITQTPYKVSISGTTVILTCPQYPGSEILWQHNDKNIGGDEDDKNIGSDEDHLSLKEFSELEQSGYYVCYPRGSKPEDANFYLYLRARVCENCMEMDVMSVATIVIVDICITGGLLLLVYYWS

SEQ ID NO: 65 - protein, 21 aa, Artificial Sequence
  MLB014.SP (i.e. the signal peptide of CD3ζ)
MKWKALFTAAILQAQLPITEA

SEQ ID NO: 66 - protein, 9 aa, Artificial Sequence
  MLB014.EM
QSFGLLDPK

SEQ ID NO: 67 - protein, 21 aa, Artificial Sequence
  MLB014.TM(i.e. the transmembrane domain of CD3ζ)
LCYLLDGILFIYGVILTALFL

SEQ ID NO: 68 - protein, 22 aa, Artificial Sequence
  MLB046.SP  (i.e. the signal peptide of CD3ε)
MQSGTHWRVLGLCLLSVGVWGQ

SEQ ID NO: 69 - protein, 104 aa, Artificial Sequence
  MLB046.EM(i.e. the extracellular domain of CD3ε)
DGNEEMGGITQTPYKVSISGTTVILTCPQYPGSEILWQHNDKNIGGDEDDKNIGSDEDHLSLKEFSELEQSGYYVCYPRGSKPEDANFYLYLRARVCENCMEMD

SEQ ID NO: 70 - protein, 26 aa, Artificial Sequence
  MLB046.TM(i.e. the transmembrane domain of CD3ε)
VMSVATIVIVDICITGGLLLLVYYWS

SEQ ID NO: 71 - protein, 152 aa, Artificial Sequence; identical to SEQ ID NO: 64
  LG212 *(CD3ε.△IC)

SEQ ID NO: 72 - DNA, 1733 bp, Artificial Sequence
  CAG promoter
ctcgacattgattattgactagttattaatagtaatcaattacggggtcattagttcatagcccatatatggagttccgcgttacataacttacggtaaatggcccgcctggctgaccgcccaacgacccccgcccattgacgtcaataatgacgtatgttcccatagtaacgccaatagggactttccattgacgtcaatgggtggagtatttacggtaaactgcccacttggcagtacatcaagtgtatcatatgccaagtacgccccctattgacgtcaatgacggtaaatggcccgcctggcattatgcccagtacatgaccttatgggactttcctacttggcagtacatctacgtattagtcatcgctattaccatggtcgaggtgagccccacgttctgcttcactctccccatctcccccccctccccacccccaattttgtatttatttattttttaattattttgtgcagcgatgggggcggggggggggggggggcgcgcgccaggcggggcggggcggggcgaggggcggggcggggcgaggcggagaggtgcggcggcagccaatcagagcggcgcgctccgaaagtttccttttatggcgaggcggcggcggcggcggccctataaaaagcgaagcgcgcggcgggcgggagtcgctgcgcgctgccttcgccccgtgccccgctccgccgccgcctcgcgccgcccgccccggctctgactgaccgcgttactcccacaggtgagcgggcgggacggcccttctcctccgggctgtaattagcgcttggtttaatgacggcttgtttcttttctgtggctgcgtgaaagccttgaggggctccgggagggccctttgtgcggggggagcggctcggggggtgcgtgcgtgtgtgtgtgcgtggggagcgccgcgtgcggctccgcgctgcccggcggctgtgagcgctgcgggcgcggcgcggggctttgtgcgctccgcagtgtgcgcgaggggagcgcggccgggggcggtgccccgcggtgcggggggggctgcgaggggaacaaaggctgcgtgcggggtgtgtgcgtgggggggtgagcagggggtgtgggcgcgtcggtcgggctgcaaccccccctgcacccccctccccgagttgctgagcacggcccggcttcgggtgcggggctccgtacggggcgtggcgcggggctcgccgtgccgggcggggggtggcggcaggtgggggtgccgggcggggcggggccgcctcgggccggggagggctcgggggaggggcgcggcggcccccggagcgccggcggctgtcgaggcgcggcgagccgcagccattgccttttatggtaatcgtgcgagagggcgcagggacttcctttgtcccaaatctgtgcggagccgaaatctgggaggcgccgccgcaccccctctagcgggcgcggggcgaagcggtgcggcgccggcaggaaggaaatgggcggggagggccttcgtgcgtcgccgcgccgccgtccccttctccctctccagcctcggggctgtccgcggggggacggctgccttcgggggggacggggcagggcggggttcggcttctggcgtgtgaccggcggctctagagcctctgctaaccatgttcatgccttcttctttttcctacagctcctgggcaacgtgctggttattgtgctgtctcatcattttggcaaagaattg

SEQ ID NO: 73 - protein, 514 aa, Artificial Sequence
  LG222*
MALPVTALLLPLALLLHAARPEVQLVESGGGLVQPGGSLKLSCAASGFTFNKYAMNWVRQAPGKGLEWVARIRSKYNNYATYYADSVKDRFTISRDDSKNTAYLQMNNLKTEDTAVYYCVRHGNFGNSYISYWAYWGQGTLVTVSSGGGGSGGGGSGGGGSGGGGSQTVVTQEPSLTVSPGGTVTLTCGSSTGAVTSGYYPNWVQQKPGQAPRGLIGGTKFLAPGTPARFSGSLLGGKAALTLSGVQPEDEAEYYCALWYSNRWVFGGGTKLTVLQSFGLLDPKLCYLLDGILFIYGVILTALFLRVKFSRSADYSARRLRNARAQSRKQRQLKADAKKAIGRLQLRTLKQGDKEIGPDGDSCAVCIELYKPNDLVRILTCNHIFHKTCVDPWLLEHRTCPMCKCDILKALGIEVDVEDGSVSLQVPVSNEISNSASSHEEDNRSETASSGYASVQGTDEPPLEEHVQSTNESLQLVNHEANSVAVDVIPHVDNPTFEEDETPNQETAVREIKS

SEQ ID NO: 74 - protein, 551 aa, Artificial Sequence
  LG222.1*
MALPVTALLLPLALLLHAARPEVQLVESGGGLVQPGGSLKLSCAASGFTFNKYAMNWVRQAPGKGLEWVARIRSKYNNYATYYADSVKDRFTISRDDSKNTAYLQMNNLKTEDTAVYYCVRHGNFGNSYISYWAYWGQGTLVTVSSGGGGSGGGGSGGGGSGGGGSQTVVTQEPSLTVSPGGTVTLTCGSSTGAVTSGYYPNWVQQKPGQAPRGLIGGTKFLAPGTPARFSGSLLGGKAALTLSGVQPEDEAEYYCALWYSNRWVFGGGTKLTVLGTTTPAPRPPTPAPTIASQPLSLRPEACRPAAGGAVHTRGLDFACDIYIWAPLAGTCGVLLLSLVITRVKFSRSADYSARRLRNARAQSRKQRQLKADAKKAIGRLQLRTLKQGDKEIGPDGDSCAVCIELYKPNDLVRILTCNHIFHKTCVDPWLLEHRTCPMCKCDILKALGIEVDVEDGSVSLQVPVSNEISNSASSHEEDNRSETASSGYASVQGTDEPPLEEHVQSTNESLQLVNHEANSVAVDVIPHVDNPTFEEDETPNQETAVREIKS

SEQ ID NO: 75 - protein, 529 aa, Artificial Sequence
  LG222.2*
MALPVTALLLPLALLLHAARPEVQLVESGGGLVQPGGSLKLSCAASGFTFNKYAMNWVRQAPGKGLEWVARIRSKYNNYATYYADSVKDRFTISRDDSKNTAYLQMNNLKTEDTAVYYCVRHGNFGNSYISYWAYWGQGTLVTVSSGGGGSGGGGSGGGGSGGGGSQTVVTQEPSLTVSPGGTVTLTCGSSTGAVTSGYYPNWVQQKPGQAPRGLIGGTKFLAPGTPARFSGSLLGGKAALTLSGVQPEDEAEYYCALWYSNRWVFGGGTKLTVLDSGQVLLESNIKVLPTWSTPVQPMALIVLGGVAGLLLFIGLGIFFRVKFSRSADYSARRLRNARAQSRKQRQLKADAKKAIGRLQLRTLKQGDKEIGPDGDSCAVCIELYKPNDLVRILTCNHIFHKTCVDPWLLEHRTCPMCKCDILKALGIEVDVEDGSVSLQVPVSNEISNSASSHEEDNRSETASSGYASVQGTDEPPLEEHVQSTNESLQLVNHEANSVAVDVIPHVDNPTFEEDETPNQETAVREIKS

SEQ ID NO: 76 - protein, 204 aa, Artificial Sequence
  GRAIL.IC.ZF mutant (Zinc-finger→CD8a hinge)
YSARRLRNARAQSRKQRQLKADAKKAIGRLQLRTLKQGDKEIGPDGDSGTTTPAPRPPTPAPTIASQPLSLRPEACRPAAGGAVHTRGLDFACDCDILKALGIEVDVEDGSVSLQVPVSNEISNSASSHEEDNRSETASSGYASVQGTDEPPLEEHVQSTNESLQLVNHEANSVAVDVIPHVDNPTFEEDETPNQETAVREIKS

SEQ ID NO: 77 - protein, 200 aa, Artificial Sequence
  GRAIL.IC.H2N2 mutant
YSARRLRNARAQSRKQRQLKADAKKAIGRLQLRTLKQGDKEIGPDGDSCAVCIELYKPNDLVRILTCNRIFRKTCVDPWLLEHRTCPMCKCDILKALGIEVDVEDGSVSLQVPVSNEISNSASSHEEDNRSETASSGYASVQGTDEPPLEEHVQSTNESLQLVNHEANSVAVDVIPHVDNPTFEEDETPNQETAVREIKS

SEQ ID NO: 78 - protein, 376 aa, Artificial Sequence
  RNF133
MHLLKVGTWRNNTASSWLMKFSVLWLVSQNCCRASVVWMAYMNISFHVGNHVLSELGETGVFGRSSTLKRVAGVIVPPEGKIQNACNPNTIFSRSKYSETWLALIERGGCTFTQKIKVATEKGASGVIIYNVPGTGNQVFPMFHQAFEDVVVVMIGNLKGTEIFHLIKKGVLITAVVEVGRKHIIWMNHYLVSFVIVTTATLAYFIFYHIHRLCLARIQNRRWQRLTTDLQNTFGQLQLRVVKEGDEEINPNGDSCVICFERYKPNDIVRILTCKHFFHKNCIDPWILPHGTCPICKCDILKVLGIQVVVENGTEPLQVLMSNELPETLSPSEEETNNEVSPAGTSDKVIHVEENPTSQNNDIQPHSVVEDVHPSP

SEQ ID NO: 79 - protein, 166 aa, Artificial Sequence
  RNF133.IC
HRLCLARIQNRRWQRLTTDLQNTFGQLQLRVVKEGDEEINPNGDSCVICFERYKPNDIVRILTCKHFFHKNCIDPWILPHGTCPICKCDILKVLGIQVVVENGTEPLQVLMSNELPETLSPSEEETNNEVSPAGTSDKVIHVEENPTSQNNDIQPHSVVEDVHPSP

SEQ ID NO: 80 - protein, 155 aa, Artificial Sequence
  RNF122
MHPFQWCNGCFCGLGLVSTNKSCSMPPISFQDLPLNIYMVIFGTGIFVFMLSLIFCCYFISKLRNQAQSERYGYKEVVLKGDAKKLQLYGQTCAVCLEDFKGKDELGVLPCQHAFHRKCLVKWLEVRCVCPMCNKPIASPSEATQNIGILLDELV

SEQ ID NO: 81 - protein, 95 aa, Artificial Sequence
  RNF122.rIC
SKLRNQAQSERYGYKEVVLKGDAKKLQLYGQTCAVCLEDFKGKDELGVLPCQHAFHRKCLVKWLEVRCVCPMCNKPIASPSEATQNIGILLDELV

SEQ ID NO: 82 - protein, 203 aa, Artificial Sequence
  RNF152
METLSQDSLLECQICFNYYSPRRRPKLLDCKHTCCSVCLQQMRTSQKDVRCPWCRGVTKLPPGFSVSQLPDDPEVLAVIAIPHTSEHTPVFIKLPSNGCYMLPLPISKERALLPGDMGCRLLPGSQQKSVTVVTIPAEQQPLQGGAPQEAVEEEQDRRGVVKSSTWSGVCTVILVACVLVFLLGIVLHNMSCISKRFTVISCG

SEQ ID NO: 83 - protein, 165 aa, Artificial Sequence
  RNF152.rIC
WTSSKVVGRRDQEEEVAEQPAGGQLPQQEAPITVVTVSKQQSGPLLRCGMDGPLLAREKSIPLPLMYCGNSPLKIFVPTHESTHPIAIVALVEPDDPLQSVSFGPPLKTVGRCWPCRVDKQSTRMQQLCVSCCTHKCDLLKPRRRPSYYNFCIQCELLSDQSLTE

SEQ ID NO: 84 - protein, 42 aa, Artificial Sequence
  GRAIL- zinc-finger domain
CAVCIELYKPNDLVRILTCNHIFHKTCVDPWLLEHRTCPMCK

SEQ ID NO: 85 - protein, 46 aa, Artificial Sequence; identical to SEQ ID NO: 16
  CD8  hinge

SEQ ID NO: 86 - protein, 544 aa, Artificial Sequence
  LG116*
MALPVTALLLPLALLLHAARPQVQLVQSGGGVVQPGRSLRLSCKASGYTFTRYTMHWVRQAPGKGLEWIGYINPSRGYTNYNQKFKDRFTISRDNSKNTAFLQMDSLRPEDTGVYFCARYYDDHYSLDYWGQGTPVTVSSGGGGSGGGGSGGGGSDIQMTQSPSSLSASVGDRVTITCSASSSVSYMNWYQQTPGKAPKRWIYDTSKLASGVPSRFSGSGSGTDYTFTISSLQPEDIATYYCQQWSSNPFTFGQGTKLQITRGSGSGSGSVNISGQNTMNMVKVPECRLADELGGLWENSRFTDCCLCVAGQEFQAHKAILAARSPVFSAMFEHEMEESKKNRVEINDVEPEVFKEMMCFIYTGKAPNLDKMADDLLAAADKYALERLKVMCEDALCSNLSVENAAEILILADLHSADQLKTQAVDFINYHASDVLETSGWKSMVVSHPHLVAEAYRSLASAQCPFLGPPRKRLKQSGTTTPAPRPPTPAPTIASQPLSLRPEACRPAAGGAVHTRGLDFACDIYIWAPLAGTCGVLLLSLVIT

SEQ ID NO: 87 - protein, 525 aa, Artificial Sequence
  LG118*
MALPVTALLLPLALLLHAARPEVQLVESGGGLVQPGGSLKLSCAASGFTFNKYAMNWVRQAPGKGLEWVARIRSKYNNYATYYADSVKDRFTISRDDSKNTAYLQMNNLKTEDTAVYYCVRHGNFGNSYISYWAYWGQGTLVTVSSGGGGSGGGGSGGGGSGGGGSQTVVTQEPSLTVSPGGTVTLTCGSSTGAVTSGYYPNWVQQKPGQAPRGLIGGTKFLAPGTPARFSGSLLGGKAALTLSGVQPEDEAEYYCALWYSNRWVFGGGTKLTVLGSGSGSGRLNFGDDIPSALRIAKKKRWNSIEERRIHQESELHSYLSRLIAAERERELEECQRNHEGDEDDSHVRAQQACIEAKHDKYMADMDELFSQVDEKRKKRDIPDYLCGKISFELMREPCITPSGITYDRKDIEEHLQRVGHFDPVTRSPLTQEQLIPNLAMKEVIDAFISENGWVEDYGTTTPAPRPPTPAPTIASQPLSLRPEACRPAAGGAVHTRGLDFACDIYIWAPLAGTCGVLLLSLVIT

SEQ ID NO: 88 - DNA, 1149 bp, Artificial Sequence
  EF1α promotor
gggcagagcgcacatcgcccacagtccccgagaagttggggggaggggtcggcaattgaaccggtgcctagagaaggtggcgcggggtaaactgggaaagtgatgtcgtgtactggctccgcctttttcccgagggtgggggagaaccgtatataagtgcagtagtcgccgtgaacgttctttttcgcaacgggtttgccgccagaacacaggtaagtgccgtgtgtggttcccgcgggcctggcctctttacgggttatggcccttgcgtgccttgaattacttccacgcccctggctgcagtacgtgattcttgatcccgagcttcgggttggaagtgggtgggagagttcgaggccttgcgcttaaggagccccttcgcctcgtgcttgagttgaggcctggcctgggcgctggggccgccgcgtgcgaatctggtggcaccttcgcgcctgtctcgctgctttcgataagtctctagccatttaaaatttttgatgacctgctgcgacgctttttttctggcaagatagtcttgtaaatgcgggccaagatctgcacactggtatttcggtttttggggccgcgggcggcgacggggcccgtgcgtcccagcgcacatgttcggcgaggcggggcctgcgagcgcggccaccgagaatcggacgggggtagtctcaagctggccggcctgctctggtgcctggcctcgcgccgccgtgtatcgccccgccctgggcggcaaggctggcccggtcggcaccagttgcgtgagcggaaagatggccgcttcccggccctgctgcagggagctcaaaatggaggacgcggcgctcgggagagcgggcgggtgagtcacccacacaaaggaaaagggcctttccgtcctcagccgtcgcttcatgtgactccacggagtaccgggcgccgtccaggcacctcgattagttcttttggagtacgtcgtctttaggttggggggaggggttttatgcgatggagtttccccacactgagtgggtggagactgaagttaggccagcttggcacttgatgtaattctccttggaatttgccctttttgagtttggatcttggttcattctcaagcctcagacagtggttcaaagtttttttcttccatttcag

SEQ ID NO: 89 - protein, 30 aa, Artificial Sequence
  CD3ζ transmembrane domain variant(used in LG222,i.e. CD3ζ.ΔIC-1)
QSFGLLDPKLCYLLDGILFIYGVILTALFL

SEQ ID NO: 90 - protein, 9 aa, Artificial Sequence
  Intracellular domain (used in LG222, LG222.1, LG222.2)
RVKFSRSAD

SEQ ID NO: 91 - protein, 7 aa, Artificial Sequence
  Linker between scFv and E3 ligase or between CD8 TM and E3 ligase
GSGSGSG